European Patent Application EP 4 230 196 A1, published August 23, 2023. Title: COMPOUNDS FOR USE IN THE TREATMENT OF DYSTROPHINOPATHIES. Applicant: SOM INNOVATION BIOTECH, S. A. Regents of the University of Minnesota. The sequence listing filed with the application follows.

SEQUENCE LISTING (4 sequences)

SEQ ID NO: 1 - DNA, 24 bp, Artificial Sequence
  Primer Utro-F1
cctgatgatgggcagaacgaattc

SEQ ID NO: 2 - DNA, 24 bp, Artificial Sequence
  Primer Utro-R1
ctgatgggtggtttcccactcttg

SEQ ID NO: 3 - DNA, 24 bp, Artificial Sequence
  Primer 18S-F1
cgcacggccggtacagtgaaactg

SEQ ID NO: 4 - DNA, 24 bp, Artificial Sequence
  Primer 18S-R1
cacccgtggtcaccatggtaggca